European Patent Specification EP 3 835 411 B9, published October 4, 2023. Title: Recombinant yeast, construction method and application thereof in preparation of tyrosol and derivatives. Applicant: Yantai Huakang Rongzan Biotechnology Co., Ltd. The sequence listing filed with the application follows.

SEQUENCE LISTING (44 sequences)

SEQ ID NO: 1 - protein, 825 aa, Bifidobacterium adolescentis
MTSPVIGTPWKKLNAPVSEEAIEGVDKYWRAANYLSIGQIYLRSNPLMKEPFTREDVKHRLVGHWGTTPGLNFLIGHINRLIADHQQNTVIIMGPGHGGPAGTAQSYLDGTYTEYFPNITKDEAGLQKFFRQFSYPGGIPSHYAPETPGSIHEGGELGYALSHAYGAVMNNPSLFVPAIVGDGEAETGPLATGWQSNKLINPRTDGIVLPILHLNGYKIANPTILSRISDEELHEFFHGMGYEPYEFVAGFDNEDHLSIHRRFAELFETVFDEICDIKAAAQTDDMTRPFYPMIIFRTPKGWTCPKFIDGKKTEGSWRSHQVPLASARDTEAHFEVLKNWLESYKPEELFDENGAVKPEVTAFMPTGELRIGENPNANGGRIREELKLPKLEDYEVKEVAEYGHGWGQLEATRRLGVYTRDIIKNNPDSFRIFGPDETASNRLQAAYDVTNKQWDAGYLSAQVDEHMAVTGQVTEQLSEHQMEGFLEGYLLTGRHGIWSSYESFVHVIDSMLNQHAKWLEATVREIPWRKPISSMNLLVSSHVWRQDHNGFSHQDPGVTSVLLNKCFNNDHVIGIYFPVDSNMLLAVAEKCYKSTNKINAIIAGKQPAATWLTLDEARAELEKGAAEWKWASNVKSNDEAQIVLAATGDVPTQEIMAAADKLDAMGIKFKVVNVVDLVKLQSAKENNEALSDEEFAELFTEDKPVLFAYHSYARDVRGLIYDRPNHDNFNVHGYEEQGSTTTPYDMVRVNNIDRYELQAEALRMIDADKYADKINELEAFRQEAFQFAVDNGYDHPDYTDWVYSGVNTNKQGAISATAATAGDNE

SEQ ID NO: 2 - protein, 825 aa, Bifidobacterium breve
MTSPVIGTPWKKLNAPVSEESLEGVDKYWRVANYLSIGQIYLRSNPLMKAPFTREDVKHRLVGHWGTTPGLNFLIGHINRFIADHGQNTVIIMGPGHGGPAGTSQSYLDGTYTETFPKITKDEAGLQKFFRQFSYPGGIPSHFAPETPGSIHEGGELGYALSHAYGAIMDNPSLFVPAIVGDGEAETGPLATGWQSNKLVNPRTDGIVLPILHLNGYKIANPTILSRISDEELHEFFHGMGYEPYEFVAGFDDEDHMSIHRRFAELWETIWDEICDIKAAAQTDNVHRPFYPMLIFRTPKGWTCPKYIDGKKTEGSWRAHQVPLASARDTEAHFEVLKNWLESYKPEELFDANGAVKDDVLAFMPKGELRIGANPNANGGVIRDDLKLPNLEDYEVKEVAEYGHGWGQLEATRTLGAYTRDIIRNNPRDFRIFGPDETASNRLQASYEVTNKQWDAGYISDEVDEHMHVSGQVVEQLSEHQMEGFLEAYLLTGRHGIWSSYESFVHVIDSMLNQHAKWLEATVREIPWRKPIASMNLLVSSHVWRQDHNGFSHQDPGVTSVLLNKCFHNDHVIGIYFATDANMLLAIAEKCYKSTNKINAIIAGKQPAATWLTLDEARAELAKGAAAWDWASTAKNNDEAEVVLAAAGDVPTQEIMAASDKLKELGVKFKVVNVADLLSLQSAKENDEALSDEEFADIFTADKPVLFAYHSYAHDVRGLIYDRPNHDNFNVHGYEEEGSTTTPYDMVRVNRIDRYELTAEALRMIDADKYADKIDELEKFRDEAFQFAVDKGYDHPDYTDWVYSGVNTDKKGAVTATAATAGDNE

SEQ ID NO: 3 - DNA, 2478 bp, Artificial sequence
atgacctctccagttattggtactccatggaaaaaattgaacgccccagtttctgaagaggctattgaaggtgttgataagtattggagagctgccaactatttgtccattggtcaaatctacttgaggtctaacccattgatgaaggaaccattcactagggaagatgttaagcacagattggttggtcattggggtactactccaggtttgaattttttgatcggtcacatcaacagattgatcgctgatcatcaacaaaacaccgttattatcatgggtccaggtcatggtggtccagctggtactgctcaatcttatttggatggtacttacaccgaatacttcccaaacattactaaggatgaagctggcttgcaaaagttcttcagacaattttcttacccaggtggtatcccatctcattatgctccagaaacaccaggttctattcatgaaggtggtgaattgggttatgctttgtctcatgcttatggtgctgttatgaacaacccatctttgtttgttccagctatagttggtgatggtgaagctgaaactggtccattggctactggttggcaatctaacaaattgattaacccaagaaccgacggtatcgttttgccaattttacatttgaacggttacaagatcgctaacccaaccattttgtccagaatctctgatgaagaattgcacgaattcttccatggtatgggttatgaaccatacgaatttgttgctggtttcgacaacgaagatcatttgtctatccatagaagattcgccgagttgttcgaaactgttttcgacgaaatttgcgatattaaggctgctgctcaaactgatgatatgactagaccattttaccccatgatcattttcagaactccaaaaggttggacctgtccaaagtttatcgatggtaaaaagactgaaggctcttggagatctcatcaagttccattggcatctgctagagatactgaagctcatttcgaagttttgaagaactggttggaaagctacaaacctgaagagttgtttgacgaaaatggtgcagttaagcctgaagttactgcttttatgccaacaggtgaattgagaattggtgaaaatccaaatgctaacggtggtagaatcagggaagaattgaaattgccaaagttggaagattacgaggtcaaagaagttgctgaatacggtcatggttggggtcaattggaagctactagaagattgggtgtttacaccagagacatcatcaagaacaatccagactccttcagaatttttggtccagacgaaactgcttctaacagattgcaagctgcttacgatgttaccaacaaacaatgggatgctggttatttgtctgcccaagttgatgaacatatggctgttactggtcaagttaccgaacaattgtcagaacatcaaatggaaggtttcttggagggttacttgttgactggtagacatggtatttggtcctcttacgaatctttcgttcacgttatcgactctatgttgaatcaacacgctaagtggttagaagctaccgttagagaaattccttggagaaagccaatctcctctatgaacttgttggtttcttcacacgtttggagacaagatcataacggtttttcacatcaagatccaggtgttacttctgtcttgttgaacaagtgtttcaacaacgatcatgtcatcggtatctacttcccagttgactctaatatgttgttggctgttgctgaaaagtgctacaaatctaccaacaagatcaacgctattatcgctggtaagcaaccagctgctacttggttgactttagatgaagctagagctgaattggaaaaaggtgctgctgaatggaaatgggcttctaatgttaagtccaacgatgaagctcaaatcgttttggctgctacaggtgatgttccaactcaagaaattatggctgcagctgataagttggatgctatgggtattaagttcaaggttgttaacgttgtcgacctggttaagttgcaatcagctaaagaaaacaacgaagccttgtccgacgaagaatttgctgagttgtttactgaagataagccagttttgttcgcctaccattcttacgctagagatgttagaggtttgatatacgatagaccaaaccacgataacttcaacgttcatggttatgaagaacaaggttctactactaccccatacgatatggttagagttaacaacatcgacaggtacgaattacaagctgaagccttgagaatgattgatgcagataagtacgccgacaagattaacgaactagaagcttttagacaagaggcctttcaattcgctgttgataatggttacgatcacccagattataccgattgggtttattctggtgtcaacactaacaagcaaggtgctatttctgctactgctgcaactgctggtgataatgaataa

SEQ ID NO: 4 - DNA, 2475 bp, Artificial sequence
atgacctctccagttattggtactccatggaaaaaattgaacgccccagtttctgaagaatccttggaaggtgttgataagtattggagagttgccaactacttgtccattggtcaaatctacttgaggtctaacccattgatgaaggctccattcactagagaagatgttaagcacagattggttggtcattggggtactactccaggtttgaattttttgatcggtcacatcaacagattcattgctgatcatggtcaaaacaccgttattatcatgggtccaggtcatggtggtccagctggtacttctcaatcttatttggatggtacttacaccgagactttcccaaagattacaaaagatgaagctggcttgcagaagttcttcagacaattttcttatccaggtggtatcccatctcattttgctccagaaacaccaggttctattcatgaaggtggtgaattgggttatgctttgtctcatgcttatggtgccattatggataacccatctttgtttgttccagccatagttggtgatggtgaagctgaaactggtccattggctactggttggcaatctaacaaattggttaacccaagaaccgatggtatcgttttgccaatcttgcatttgaacggttacaagattgctaacccaaccatcttgtccagaatctctgatgaagaattgcatgagttcttccatggtatgggttatgaaccatacgaatttgttgctggtttcgatgatgaagatcacatgtccattcatagaagattcgctgaattgtgggaaaccatttgggacgaaatttgcgatattaaggctgctgctcaaaccgataatgttcatagaccattttaccccatgctgattttcagaactccaaaaggttggacttgcccaaagtacattgatggtaaaaagactgaaggttcttggagagcacatcaagttccattggcatctgctagagatactgaagctcatttcgaagttttgaagaactggttggaaagctacaaacctgaagagttgtttgatgctaatggtgctgttaaggatgatgttttggcttttatgccaaagggtgaattgagaattggtgctaatccaaatgcaaacggtggtgttattagagatgatctgaagttgccaaacttggaagattacgaagtcaaagaagttgccgaatacggtcatggttggggtcaattggaagctactagaactttgggtgcttacaccagagatatcattagaaacaacccaagagacttcagaattttcggtccagacgaaactgcttctaatagattgcaagcttcttacgaggttaccaacaaacaatgggatgctggttacatttccgatgaagttgatgaacatatgcacgtttctggtcaagttgtcgaacaattgtcagaacatcaaatggaaggttttttggaggcttacttgttgactggtagacatggtatttggtcctcttacgaatctttcgttcacgttatcgactctatgttgaatcaacacgctaaatggttggaagccaccgttagagaaattccttggagaaaacctattgcctccatgaacttgttggtttcttcacatgtttggagacaagatcacaacggtttctctcatcaagatccaggtgttacttctgtcttgttgaacaagtgtttccacaacgatcatgtcatcggtatctactttgctactgatgctaacatgttgttggctattgctgaaaagtgttacaagtccaccaacaagattaacgctattattgctggtaaacaaccagctgctacttggttgactttggatgaagctagagctgaattggctaaaggtgctgctgcttgggattgggcttctactgctaaaaacaatgatgaagccgaagttgttttagctgctgctggtgatgttccaactcaagaaattatggctgcttccgacaagttgaaagaattgggtgttaagttcaaggttgttaacgttgccgatttgttgtcattgcaatccgctaaagaaaacgacgaagctttgtcagacgaagaatttgctgatatcttcactgctgataagccagttttgttcgcttatcattcttacgcccatgatgtcagaggtttgatatacgatagaccaaaccacgataacttcaacgttcatggttatgaagaagaaggttctactactaccccatacgatatggttagagttaacagaatcgacaggtacgaattgactgctgaagctttgagaatgattgatgcagataagtacgccgataagatcgacgaattggaaaagttcagagatgaagcctttcaattcgcagttgataagggttatgatcacccagattataccgattgggtttactctggtgttaataccgataagaaaggtgcagttactgctactgctgcaacagctggtgataatgaa

SEQ ID NO: 5 - DNA, 50 bp, Artificial sequence
atatttccgcattcatccttcaattgtgtttaaagattacggatatttaa

SEQ ID NO: 6 - DNA, 47 bp, Artificial sequence
accaataactggagaggtcatttttagtttatgtatgtgttttttgt

SEQ ID NO: 7 - DNA, 50 bp, Artificial sequence
gctatacgaagttattaggtgatatatgttatatagtctttttatttatg

SEQ ID NO: 8 - DNA, 20 bp, Artificial sequence
ctatgttcactctggcgtgc

SEQ ID NO: 9 - DNA, 50 bp, Artificial sequence; identical to SEQ ID NO: 5

SEQ ID NO: 10 - DNA, 47 bp, Artificial sequence; identical to SEQ ID NO: 6

SEQ ID NO: 11 - DNA, 50 bp, Artificial sequence
tgcaactgctggtgataatgaataagtctgaagaatgaatgatttgatga

SEQ ID NO: 12 - DNA, 46 bp, Artificial sequence
cattatacgaagttatattaagggttattcgaactgcccattcagc

SEQ ID NO: 13 - DNA, 47 bp, Artificial sequence
acaaaaaacacatacataaactaaaaatgacctctccagttattggt

SEQ ID NO: 14 - DNA, 50 bp, Artificial sequence
tcatcaaatcattcattcttcagacttattcattatcaccagcagttgca

SEQ ID NO: 15 - DNA, 47 bp, Artificial sequence; identical to SEQ ID NO: 13

SEQ ID NO: 16 - DNA, 50 bp, Artificial sequence
tcatcaaatcattcattcttcagacttattcattatcaccagctgttgca

SEQ ID NO: 17 - DNA, 46 bp, Artificial sequence
gctgaatgggcagttcgaataacccttaatataacttcgtataatg

SEQ ID NO: 18 - DNA, 50 bp, Artificial sequence
cataaataaaaagactatataacatatatcacctaataacttcgtatagc

SEQ ID NO: 19 - DNA, 24 bp, Artificial sequence
ctccgtttatgataagatgatggc

SEQ ID NO: 20 - DNA, 21 bp, Artificial sequence
gttaattgcctccgcatctaa

SEQ ID NO: 21 - protein, 520 aa, E Coli.
MKPEDFRASTQRPFTGEEYLKSLQDGREIYIYGERVKDVTTHPAFRNAAASVAQLYDALHKPEMQDSLCWNTDTGSGGYTHKFFRVAKSADDLRHERDAIAEWSRLSYGWMGRTPDYKAAFGCALGGTPGFYGQFEQNARNWYTRIQETGLYFNHAIVNPPIDRHLPTDKVKDVYIKLEKETDAGIIVSGAKVVATNSALTHYNMIGFGSAQVMGENPDFALMFVAPMDADGVKLISRASYEMVAGATGSPYDYPLSSRFDENDAILVMDNVLIPWENVLLYRDFDRCRRWTMEGGFARMYPLQACVRLAVKLDFITALLKKSLECTGTLEFRGVQADLGEVVAWRNTFWALSDSMCSEATPWVNGAYLPDHAALQTYRVLAPMAYAKIKNIIERNVTSGLIYLPSSARDLNNPQIDQYLAKYVRGSNGMDHVQRIKILKLMWDAIGSEFGGRHELYEINYSGSQDEIRLQCLRQAQSSGNMDKMMAMVDRCLSEYDQNGWTVPHLHNNDDINMLDKLLK

SEQ ID NO: 22 - protein, 170 aa, E Coli.
MQLDEQRLRFRDAMASLSAAVNIITTEGDAGQCGITATAVCSVTDTPPSLMVCINANSAMNPVFQGNGKLCVNVLNHEQELMARHFAGMTGMAMEERFSLSCWQKGPLAQPVLKGSLASLEGEIRDVQAIGTHLVYLVEIKNIILSAEGHGLIYFKRRFHPVMLEMEAAI

SEQ ID NO: 23 - DNA, 1563 bp, Artificial sequence
atgaaaccagaagatttccgcgccagtacccaacgtccgttcaccggggaagagtatctgaaaagcctgcaggatggtcgcgagatctatatctatggcgagcgagtgaaagacgtcactactcatccggcatttcgtaatgcggctgcgtctgttgcccaactgtacgacgcgctacacaaaccggagatgcaggactctctgtgctggaacaccgacaccggcagcggcggctatacccataaattcttccgcgtggcgaaaagtgccgacgacctgcgccacgaacgcgatgccatcgctgagtggtcacgcctgagctatggctggatgggccgtaccccagactacaaagctgctttcggttgcgcactgggcggaactccgggcttttacggtcagttcgagcagaacgcccgtaactggtacacccgtattcaggaaactggcctctactttaaccacgcgattgttaacccaccgatcgatcgtcatttgccgaccgataaagtaaaagacgtttacatcaagctggaaaaagagactgacgccgggattatcgtcagcggtgcgaaagtggttgccaccaactcggcgctgactcactacaacatgattggcttcggctcggcacaagtaatgggcgaaaacccggacttcgcactgatgttcgttgcgccaatggatgccgatggcgtcaaattaatctcccgcgcctcttatgagatggtcgcgggtgctaccggctcaccgtatgactacccgctctccagccgcttcgatgagaacgatgcgattctggtgatggataacgtgctgatcccatgggaaaacgtgctgctctaccgcgattttgatcgctgccgtcgctggacgatggaaggcggtttcgcccgtatgtatccgctgcaagcctgtgtgcgcctggcagtgaaactcgacttcattacggcactgctgaaaaaatcactcgaatgtaccggcaccctggagttccgtggtgtgcaggccgatctcggtgaagtggtggcgtggcgcaacaccttctgggcattgagtgactcgatgtgttctgaagcgacgccgtgggtcaacggggcttatttaccggatcatgccgcactgcaaacctatcgcgtactggcaccaatggcctacgcgaagatcaaaaacattatcgaacgcaacgttaccagtggcctgatctatctcccttccagtgcccgtgacctgaacaatccgcagatcgaccagtatctggcgaagtatgtgcgcggttcgaacggtatggatcacgtccagcgcatcaagatcctcaaactgatgtgggatgccattggcagcgagtttggtggtcgtcacgaactgtatgaaatcaactactccggtagccaggatgagattcgcctgcagtgtctgcgccaggcacaaagctccggcaatatggacaagatgatggcgatggttgatcgctgcctgtcggaatacgaccagaacggctggactgtgccgcacctgcacaacaacgacgatatcaacatgctggataagctgctgaaataa

SEQ ID NO: 24 - DNA, 513 bp, Artificial sequence
atgcaattagatgaacaacgcctgcgctttcgtgacgcaatggccagcctgtcggcagcggtaaatattatcaccaccgagggcgacgccggacaatgcgggattacggcaacggccgtctgctcggtcacggatacaccaccatcgctgatggtgtgcattaacgccaacagtgcgatgaacccggtttttcagggcaacggtaagttgtgcgtcaacgtcctcaaccatgagcaggaactgatggcacgccacttcgcgggcatgacaggcatggcgatggaagagcgttttagcctctcatgctggcaaaaaggtccgctggcgcagccggtgctaaaaggttcgctggccagtcttgaaggtgagatccgcgatgtgcaggcaattggcacacatctggtgtatctggtggagattaaaaacatcatcctcagtgcagaaggtcacggacttatctactttaaacgccgtttccatccggtgatgctggaaatggaagctgcgatttaa

SEQ ID NO: 25 - DNA, 22 bp, Artificial sequence
atgaaaccagaagatttccgcg

SEQ ID NO: 26 - DNA, 22 bp, Artificial sequence
ttatttcagcagcttatccagc

SEQ ID NO: 27 - DNA, 23 bp, Artificial sequence
atgcaattagatgaacaacgcct

SEQ ID NO: 28 - DNA, 23 bp, Artificial sequence
ttaaatcgcagcttccatttcca

SEQ ID NO: 29 - DNA, 7347 bp, Artificial sequence
tggcgaatgggacgcgccctgtagcggcgcattaagcgcggcgggtgtggtggttacgcgcagcgtgaccgctacacttgccagcgccctagcgcccgctcctttcgctttcttcccttcctttctcgccacgttcgccggctttccccgtcaagctctaaatcgggggctccctttagggttccgatttagtgctttacggcacctcgaccccaaaaaacttgattagggtgatggttcacgtagtgggccatcgccctgatagacggtttttcgccctttgacgttggagtccacgttctttaatagtggactcttgttccaaactggaacaacactcaaccctatctcggtctattcttttgatttataagggattttgccgatttcggcctattggttaaaaaatgagctgatttaacaaaaatttaacgcgaattttaacaaaatattaacgtttacaatttcaggtggcacttttcggggaaatgtgcgcggaacccctatttgtttatttttctaaatacattcaaatatgtatccgctcatgaattaattcttagaaaaactcatcgagcatcaaatgaaactgcaatttattcatatcaggattatcaataccatatttttgaaaaagccgtttctgtaatgaaggagaaaactcaccgaggcagttccataggatggcaagatcctggtatcggtctgcgattccgactcgtccaacatcaatacaacctattaatttcccctcgtcaaaaataaggttatcaagtgagaaatcaccatgagtgacgactgaatccggtgagaatggcaaaagtttatgcatttctttccagacttgttcaacaggccagccattacgctcgtcatcaaaatcactcgcatcaaccaaaccgttattcattcgtgattgcgcctgagcgagacgaaatacgcgatcgctgttaaaaggacaattacaaacaggaatcgaatgcaaccggcgcaggaacactgccagcgcatcaacaatattttcacctgaatcaggatattcttctaatacctggaatgctgttttcccggggatcgcagtggtgagtaaccatgcatcatcaggagtacggataaaatgcttgatggtcggaagaggcataaattccgtcagccagtttagtctgaccatctcatctgtaacatcattggcaacgctacctttgccatgtttcagaaacaactctggcgcatcgggcttcccatacaatcgatagattgtcgcacctgattgcccgacattatcgcgagcccatttatacccatataaatcagcatccatgttggaatttaatcgcggcctagagcaagacgtttcccgttgaatatggctcataacaccccttgtattactgtttatgtaagcagacagttttattgttcatgaccaaaatcccttaacgtgagttttcgttccactgagcgtcagaccccgtagaaaagatcaaaggatcttcttgagatcctttttttctgcgcgtaatctgctgcttgcaaacaaaaaaaccaccgctaccagcggtggtttgtttgccggatcaagagctaccaactctttttccgaaggtaactggcttcagcagagcgcagataccaaatactgtccttctagtgtagccgtagttaggccaccacttcaagaactctgtagcaccgcctacatacctcgctctgctaatcctgttaccagtggctgctgccagtggcgataagtcgtgtcttaccgggttggactcaagacgatagttaccggataaggcgcagcggtcgggctgaacggggggttcgtgcacacagcccagcttggagcgaacgacctacaccgaactgagatacctacagcgtgagctatgagaaagcgccacgcttcccgaagggagaaaggcggacaggtatccggtaagcggcagggtcggaacaggagagcgcacgagggagcttccagggggaaacgcctggtatctttatagtcctgtcgggtttcgccacctctgacttgagcgtcgatttttgtgatgctcgtcaggggggcggagcctatggaaaaacgccagcaacgcggcctttttacggttcctggccttttgctggccttttgctcacatgttctttcctgcgttatcccctgattctgtggataaccgtattaccgcctttgagtgagctgataccgctcgccgcagccgaacgaccgagcgcagcgagtcagtgagcgaggaagcggaagagcgcctgatgcggtattttctccttacgcatctgtgcggtatttcacaccgcatatatggtgcactctcagtacaatctgctctgatgccgcatagttaagccagtatacactccgctatcgctacgtgactgggtcatggctgcgccccgacacccgccaacacccgctgacgcgccctgacgggcttgtctgctcccggcatccgcttacagacaagctgtgaccgtctccgggagctgcatgtgtcagaggttttcaccgtcatcaccgaaacgcgcgaggcagctgcggtaaagctcatcagcgtggtcgtgaagcgattcacagatgtctgcctgttcatccgcgtccagctcgttgagtttctccagaagcgttaatgtctggcttctgataaagcgggccatgttaagggcggttttttcctgtttggtcactgatgcctccgtgtaagggggatttctgttcatgggggtaatgataccgatgaaacgagagaggatgctcacgatacgggttactgatgatgaacatgcccggttactggaacgttgtgagggtaaacaactggcggtatggatgcggcgggaccagagaaaaatcactcagggtcaatgccagcgcttcgttaatacagatgtaggtgttccacagggtagccagcagcatcctgcgatgcagatccggaacataatggtgcagggcgctgacttccgcgtttccagactttacgaaacacggaaaccgaagaccattcatgttgttgctcaggtcgcagacgttttgcagcagcagtcgcttcacgttcgctcgcgtatcggtgattcattctgctaaccagtaaggcaaccccgccagcctagccgggtcctcaacgacaggagcacgatcatgcgcacccgtggggccgccatgccggcgataatggcctgcttctcgccgaaacgtttggtggcgggaccagtgacgaaggcttgagcgagggcgtgcaagattccgaataccgcaagcgacaggccgatcatcgtcgcgctccagcgaaagcggtcctcgccgaaaatgacccagagcgctgccggcacctgtcctacgagttgcatgataaagaagacagtcataagtgcggcgacgatagtcatgccccgcgcccaccggaaggagctgactgggttgaaggctctcaagggcatcggtcgagatcccggtgcctaatgagtgagctaacttacattaattgcgttgcgctcactgcccgctttccagtcgggaaacctgtcgtgccagctgcattaatgaatcggccaacgcgcggggagaggcggtttgcgtattgggcgccagggtggtttttcttttcaccagtgagacgggcaacagctgattgcccttcaccgcctggccctgagagagttgcagcaagcggtccacgctggtttgccccagcaggcgaaaatcctgtttgatggtggttaacggcgggatataacatgagctgtcttcggtatcgtcgtatcccactaccgagatatccgcaccaacgcgcagcccggactcggtaatggcgcgcattgcgcccagcgccatctgatcgttggcaaccagcatcgcagtgggaacgatgccctcattcagcatttgcatggtttgttgaaaaccggacatggcactccagtcgccttcccgttccgctatcggctgaatttgattgcgagtgagatatttatgccagccagccagacgcagacgcgccgagacagaacttaatgggcccgctaacagcgcgatttgctggtgacccaatgcgaccagatgctccacgcccagtcgcgtaccgtcttcatgggagaaaataatactgttgatgggtgtctggtcagagacatcaagaaataacgccggaacattagtgcaggcagcttccacagcaatggcatcctggtcatccagcggatagttaatgatcagcccactgacgcgttgcgcgagaagattgtgcaccgccgctttacaggcttcgacgccgcttcgttctaccatcgacaccaccacgctggcacccagttgatcggcgcgagatttaatcgccgcgacaatttgcgacggcgcgtgcagggccagactggaggtggcaacgccaatcagcaacgactgtttgcccgccagttgttgtgccacgcggttgggaatgtaattcagctccgccatcgccgcttccactttttcccgcgttttcgcagaaacgtggctggcctggttcaccacgcgggaaacggtctgataagagacaccggcatactctgcgacatcgtataacgttactggtttcacattcaccaccctgaattgactctcttccgggcgctatcatgccataccgcgaaaggttttgcgccattcgatggtgtccgggatctcgacgctctcccttatgcgactcctgcattaggaagcagcccagtagtaggttgaggccgttgagcaccgccgccgcaaggaatggtgcatgcaaggagatggcgcccaacagtcccccggccacggggcctgccaccatacccacgccgaaacaagcgctcatgagcccgaagtggcgagcccgatcttccccatcggtgatgtcggcgatataggcgccagcaaccgcacctgtggcgccggtgatgccggccacgatgcgtccggcgtagaggatcgagatctcgatcccgcgaaattaatacgactcactataggggaattgtgagcggataacaattcccctctagaaataattttgtttaactttaagaaggagatataccatgggcagcagccatcatcatcatcatcacatgaaaccagaagatttccgcgccagtacccaacgtccgttcaccggggaagagtatctgaaaagcctgcaggatggtcgcgagatctatatctatggcgagcgagtgaaagacgtcactactcatccggcatttcgtaatgcggctgcgtctgttgcccaactgtacgacgcgctacacaaaccggagatgcaggactctctgtgctggaacaccgacaccggcagcggcggctatacccataaattcttccgcgtggcgaaaagtgccgacgacctgcgccacgaacgcgatgccatcgctgagtggtcacgcctgagctatggctggatgggccgtaccccagactacaaagctgctttcggttgcgcactgggcggaactccgggcttttacggtcagttcgagcagaacgcccgtaactggtacacccgtattcaggaaactggcctctactttaaccacgcgattgttaacccaccgatcgatcgtcatttgccgaccgataaagtaaaagacgtttacatcaagctggaaaaagagactgacgccgggattatcgtcagcggtgcgaaagtggttgccaccaactcggcgctgactcactacaacatgattggcttcggctcggcacaagtaatgggcgaaaacccggacttcgcactgatgttcgttgcgccaatggatgccgatggcgtcaaattaatctcccgcgcctcttatgagatggtcgcgggtgctaccggctcaccgtatgactacccgctctccagccgcttcgatgagaacgatgcgattctggtgatggataacgtgctgatcccatgggaaaacgtgctgctctaccgcgattttgatcgctgccgtcgctggacgatggaaggcggtttcgcccgtatgtatccgctgcaagcctgtgtgcgcctggcagtgaaactcgacttcattacggcactgctgaaaaaatcactcgaatgtaccggcaccctggagttccgtggtgtgcaggccgatctcggtgaagtggtggcgtggcgcaacaccttctgggcattgagtgactcgatgtgttctgaagcgacgccgtgggtcaacggggcttatttaccggatcatgccgcactgcaaacctatcgcgtactggcaccaatggcctacgcgaagatcaaaaacattatcgaacgcaacgttaccagtggcctgatctatctcccttccagtgcccgtgacctgaacaatccgcagatcgaccagtatctggcgaagtatgtgcgcggttcgaacggtatggatcacgtccagcgcatcaagatcctcaaactgatgtgggatgccattggcagcgagtttggtggtcgtcacgaactgtatgaaatcaactactccggtagccaggatgagattcgcctgcagtgtctgcgccaggcacaaagctccggcaatatggacaagatgatggcgatggttgatcgctgcctgtcggaatacgaccagaacggctggactgtgccgcacctgcacaacaacgacgatatcaacatgctggataagctgctgaaataacgcagcaggaggttaagatgcaattagatgaacaacgcctgcgctttcgtgacgcaatggccagcctgtcggcagcggtaaatattatcaccaccgagggcgacgccggacaatgcgggattacggcaacggccgtctgctcggtcacggatacaccaccatcgctgatggtgtgcattaacgccaacagtgcgatgaacccggtttttcagggcaacggtaagttgtgcgtcaacgtcctcaaccatgagcaggaactgatggcacgccacttcgcgggcatgacaggcatggcgatggaagagcgttttagcctctcatgctggcaaaaaggtccgctggcgcagccggtgctaaaaggttcgctggccagtcttgaaggtgagatccgcgatgtgcaggcaattggcacacatctggtgtatctggtggagattaaaaacatcatcctcagtgcagaaggtcacggacttatctactttaaacgccgtttccatccggtgatgctggaaatggaagctgcgattcaccaccaccaccaccactgagatccggctgctaacaaagcccgaaaggaagctgagttggctgctgccaccgctgagcaataactagcataaccccttggggcctctaaacgggtcttgaggggttttttgctgaaaggaggaactatatccggat

SEQ ID NO: 30 - protein, 824 aa, Bifidobacterium dentium
TSPVIGTPTLLLAAPVSGGAIGGVALTTAAAATLSIGGITLASAPLMLGPPTAGAVLHALVGHTGTTPGLAPLIGHIAALIAAHGGATVIIMGPGHGGPAGTAGSTLAGTTTGTPPAITLAGAGLGLPPAGPSTPGGIPSHTAPGTPGSIHGGGGLGTALSHATGAVMAAPSLPVPAIVGAGGAGTGPLATGTGSALLVAPATAGIVLPILHLAGTLIAAPTILSAISAGGLHGPPHGMGTGPTGPVAGPAAGAHLSIHAAPAGLPGTVPAGICAILAAAGTAAMTAPPTPMIIPATPLGTTCPLPIAGLLTGGSTASHGVPLASAAATGAHPGVLLATLGSTLPGGLPAAAGAVLPGVTAPMPTGGLAIGGAPAAAGGAIAGGLALPALGATGVLGVAGTGHGTGGLGATAALGVTTAAIILAAPASPAIPGPAGTASAALGAATAVTALGTAAGTLSAGVAGHMAVTGGVTGGLSGHGMGGPLGATLLTGAHGITSSTGSPVHVIASMLAGHALTLGATVAGIPTALPISSMALLVSSHVTAGAHAGPSHGAPGVTSVLLALCPAAAHVIGITPPVASAMLLAVAGLCTLSTAMIAAIIAGLGPAATTLTLAGAAAGLGLGAAGTGTASTALSAAGAGIVLASAGAVPAGGIMAAAALLAAMGILPLVVAVVALVLLGSTLGAAGAISAAAPAALPTGALPVLPATHSTAAAVAGLITAAPAHAAPAVHGTGGGGSTTTPTAMVAVAAIAATGLVAGALAMIAAALTAALIAGLGAPALGAPGPAVAAGTAHPATTATVTSGVATALGGAVSATAATAGAAG

SEQ ID NO: 31 - DNA, 2478 bp, Artificial sequence
atgacctctccagttattggtactccatggaaaaaattgaacgccccagtttctgaagaggctattgaaggtgttgataagtattggagagctgccaactatttgtccattggtcaaatctacttgaggtctaacccattgatgaaggaaccattcactagggaagatgttaagcacagattggttggtcattggggtactactccaggtttgaattttttgatcggtcacatcaacagattgatcgctgatcatcaacaaaacaccgttattatcatgggtccaggtcatggtggtccagctggtactgctcaatcttatttggatggtacttacaccgaatacttcccaaacattactaaggatgaagctggcttgcaaaagttcttcagacaattttcttacccaggtggtatcccatctcattatgctccagaaacaccaggttctattcatgaaggtggtgaattgggttatgctttgtctcatgcttatggtgctgttatgaacaacccatctttgtttgttccagctatagttggtgatggtgaagctgaaactggtccattggctactggttggcaatctaacaaattggttaacccaagaaccgatggtatcgttttgccaatcttgcatttgaacggttacaagattgctaacccaaccatcttgtccagaatctctgatgaagaattgcatgagttcttccatggtatgggttatgaaccatacgaatttgttgctggtttcgacaacgaagatcatttgtctatccatagaagattcgccgagttgttcgaaactgttttcgacgaaatttgcgatattaaggctgctgctcaaactgatgatatgactagaccattttaccccatgatcattttcagaactccaaaaggttggacctgtccaaagtttatcgatggtaaaaagactgaaggttcttggagatcacatcaagttccattggcatctgctagagatactgaagctcatttcgaagttttgaagaactggttggaaagctacaaacctgaagagttgtttgatgctaatggtgcagtaaagcctgaagttactgcttttatgccaacaggtgaattgagaattggtgaaaatccaaatgctaacggtggtagaatcagggaagaattgaatttgccagctttggaagattacgaagtcaaagaagttgctgaatacggtcatggttggggtcaattggaagctactagaagattgggtgtttacaccagagatatcatcaagaacaatccagactccttcagaatttttggtccagacgaaactgcttctaacagattgcaagctgcttacgatgttaccaacaaacaatgggatgctggttatttgtctgcccaagttgatgaacatatggctgttactggtcaagttaccgaacaattgtcagaacatcaaatggaaggttttttggaggcttacttgttgactggtagacatggtatttggtcctcttacgaatctttcgttcacgttatcgactctatgttgaatcaacacgctaaatggttggaagccactgttagagaaattccttggagaaagccaatctcctctatgaacttgttggtttcttcacacgtttggagacaagatcataacggtttctctcatcaagatccaggtgttacttccgtcttgttgaacaagtgtttcaacaacgatcatgtcatcggtatctacttcccagttgactctaatatgttgttggctgttgctgaaaagtgctacaagtctaccgatatgattaacgctattatcgctggtaagcaaccagctgctacttggttgactttagatgaagctagagctgaattggaaaaaggtgctgctgaatgggaatgggcttctactgctaaatcaaatgatgaagcccaaatcgttttggcttctgctggtgatgttccagcacaagaaattatggctgcagctgataagttggatgctatgggtattaagttcaaggttgttaacgttgtcgacctggttaagttgcaatctaccaaagaaaacgatgaagccatttccgatgcagattttgctgatttgttcaccgaagataagccagttttgttcgcttatcattcctacgctagagatgtcagaggtttgatatacgatagaccaaaccacgataacttcaacgttcatggttatgaagaacaaggttctactactaccccatacgatatggttagagttaacaacatcgacaggtatgaattggttgctgaagccttgagaatgattgatgcagataagtacgctgacaagatcgatgaattagaggcttttagaaaagaggccttccaattcgctgttgataatggttacgatcatccagattacaccgattgggtttattctggtgttaataccaacaagcaaggtgctgtttctgctactgctgctacagctggtgataatgaataa

SEQ ID NO: 32 - DNA, 47 bp, Artificial sequence; identical to SEQ ID NO: 13

SEQ ID NO: 33 - DNA, 50 bp, Artificial sequence
tcatcaaatcattcattcttcagacttattcattatcaccagctgtagca

SEQ ID NO: 34 - protein, 825 aa, Bifidobacterium animalis
MTNPVIGTPWQKLDRPVSEEAIEGMDKYWRVANYMSIGQIYLRSNPLMKEPFTRDDVKHRLVGHWGTTPGLNFLLAHINRLIADHQQNTVFIMGPGHGGPAGTAQSYIDGTYTEYYPNITKDEAGLQKFFRQFSYPGGIPSHFAPETPGSIHEGGELGYALSHAYGAIMDNPSLFVPCIIGDGEAETGPLATGWQSNKLVNPRTDGIVLPILHLNGYKIANPTILARISDEELHDFFRGMGYHPYEFVAGFDNEDHLSIHRRFAELFETIFDEICDIKAAAQTDDMTRPFYPMLIFRTPKGWTCPKFIDGKKTEGSWRAHQVPLASARDTEAHFEVLKGWMESYKPEELFNADGSIKEDVTAFMPKGELRIGANPNANGGRIREDLKLPELDQYEITGVKEYGHGWGQVEAPRSLGAYCRDIIKNNPDSFRVFGPDETASNRLNATYEVTKKQWDNGYLSALVDENMAVTGQVVEQLSEHQCEGFLEAYLLTGRHGIWSSYESFVHVIDSMLNQHAKWLEATVREIPWRKPISSVNLLVSSHVWRQDHNGFSHQDPGVTSVLLNKTFNNDHVTNIYFATDANMLLAIAEKCFKSTNKINAIFAGKQPAATWITLDEARAELEAGAAEWKWASNAKSNDEVQVVLAAAGDVPTQEIMAASDALNKMGIKFKVVNVVDLIKLQSSKENDEAMSDEDFADLFTADKPVLFAYHSYAQDVRGLIYDRPNHDNFTVVGYKEQGSTTTPFDMVRVNDMDRYALQAKALELIDADKYADKINELNEFRKTAFQFAVDNGYDIPEFTDWVYPDVKVDETSMLSATAATAGDNE

SEQ ID NO: 35 - protein, 825 aa, Bifidobacterium bifidum
MTSPVIGTPWKKLNAPVSEEALEGVDKYWRVANYLSIGQIYLRSNPLMKEPFTREDVKHRLVGHWGTTPGLNFLIGHINRFIADHGQNTVFIMGPGHGGPAGTSQSYLDGTYTETYPNITKDEAGLQKFFRQFSYPGGIPSHFAPETPGSIHEGGELGYALSHAYGAIMDNPSLFVPCIVGDGEAETGPLATGWQSNKLVNPRTDGIVLPILHLNGYKIANPTILSRISDEELHEFFHGMGYEPYEFVAGFDDEDHMSIHRRFAELFESVWDEICDIKAAANTDNMHRPFYPMIIFRTPKGWTCPKYIDGKKTEAPGAPTRVPLASARDTEAHFEVLKNWLESYKPEELFDANGAVKDDVLAFMPKGELRIGANPNANGGVIRKDLVLPALEDYEVKEVKEFGHGWGQLEATRRLGVYTRDIIKNNMHDFRIFGPDETASNRLQASYEVTNKQWDAGYISDEVDEHMHVSGQVVEQLSEHQMEGFLEAYLLTGRHGIWSSYESFVHVIDSMLNQHAKWLEATVREIPWRKPIASMNLLVSSHVWRQDHNGFSHQDPGVTSVLLNKCFHNDHVIGIYFATDANMLLAIAEKCYKSTNKINAIIAGKQPAATWLTLDEARAELAKGAAAWDWASTAKTNDEAQVVLAAAGDVPTQEIMAASDKLKALGIKFKVVNVADLLSLQSAKENDEALTDEEFADIFTADKPVLFAYHSYAHDVRGLIYDRPNHDNFNVHGYEEEGSTTTPYDMVRVNELDRYELTAEALRMIDADKYADEIQKLEDFRQEAFQFAVDKGYDHPDYTDWVYSGVKTDKKGAVTATAATAGDNE

SEQ ID NO: 36 - protein, 825 aa, Bifidobacterium lactis; identical to SEQ ID NO: 34

SEQ ID NO: 37 - protein, 825 aa, Bifidobacterium longum
MTSPVIGTPWKKLNAPVSEEALEGVDKYWRVANYLSIGQIYLRSNPLMKEPFTREDVKHRLVGHWGTTPGLNFLIGHINRFIADHGQNTVIIMGPGHGGPAGTSQSYLDGTYTETFPKITKDEAGLQKFFRQFSYPGGIPSHFAPETPGSIHEGGELGYALSHAYGAIMDNPSLFVPAIVGDGEAETGPLATGWQSNKLVNPRTDGIVLPILHLNGYKIANPTILSRISDEELHEFFHGMGYEPYEFVAGFDDEDHMSIHRRFAELWETIWDEICDIKAAAQTDNVHRPFYPMLIFRTPKGWTCPKYIDGKKTEGSWRAHQVPLASARDTEAHFEVLKNWLESYKPEELFDANGAVKDDVLAFMPKGELRIGANPNANGGVIRDDLKLPNLEDYEVKEVAEYGHGWGQLEATRTLGVYTRDIIKNNPRDFRIFGPDETASNRLQASYEVTNKQWDAGYISDEVDEHMHVSGQVVEQLSEHQMEGFLEAYLLTGRHGIWSSYESFVHVIDSMLNQHAKWLEATVREIPWRKPIASMNLLVSSHVWRQDHNGFSHQDPGVTSVLLNKCFHNDHVIGIYFATDANMLLAIAEKCYKSTNKINAIIAGKQPAATWLTLDEARAELEKGAAAWDWASTAKNNDEAEVVLAAAGDVPTQEIMAASDKLKELGVKFKVVNVVDLLSLQSAKENDEALTDEEFADIFTADKPVLFAYHSYAHDVRGLIYDRPNHDNFNVHGYEEEGSTTTPYDMVRVNRIDRYELTAEALRMIDADKYADKIDELEKFRDEAFQFAVDKGYDHPDYTDWVYSGVNTDKKGAVTATAATAGDNE

SEQ ID NO: 38 - protein, 825 aa, Bifidobacterium mongoliense
MTSPVIGTPWTKLDEPVSEETLEGIDKYWRAANYLSIGQIYLRSNPLMKEPFTRDNVKHRLVGHWGTTPGLNFLLGHINHLIAAHKQNTVIIMGPGHGGPAGTAQSYLDGTYTEYYPKITKDEAGLQKFFRQFSYPGGIPSHFAPETPGSIHEGGELGYALSHAYGAVMNNPSLFVPAIVGDGEAETGPLATGWQSNKLVNPRTDGIVLPILHLNGYKIANPSILSRISDEELHDFFHGMGYEPYEFVAGFDNEDHLSIHRRFADLFESIFDEICDIKAQAQTDDMTRPFYPMIIFRTPKGWTCPKYIDGKKTEGSWRAHQVPLASARDTEAHFEVLKHWLESYKPEELFAADGSIKPEVTSFMPEGELRIGENPNANGGRIREDLKLPKLEDYEVNEVKEYGHGWGQLEATRRMGVYTRDVIKLNPDSFRIFGPDETASNRLAAAYEVTNKQWDAGYLSAQVDEHMAVTGQVTEQLSEHQMEGFLEGYLLTGRHGVWSSYESFVHVIDSMLNQHAKWLEATVREIPWRKPISSVNLLVSSHVWRQDHNGFSHQDPGVTSVLLNKTFNNDHVVNIYFPVDANMLLAVTERCYKSTNEINAIIAGKQPAATWLTLDEARAELDKGAAEWTWASNTDNNDDVQVVLACAGDVPTQEIMAAADKLSAFGIKFKVVNVVDLLKLQSAKENDEALSDAEFSDLFTADKPVLFAYHSYAHDVRGLIYDRPNHDNFNVHGYKEQGSTTTPYDMVRVNDMDRYALTAEALRMVDKDKYAADIDKLEAFRKEAFQFAVDKGYDHPDYTDWLWHGVKSDKAGAVTATAATAGDNE

SEQ ID NO: 39 - protein, 825 aa, Bifidobacterium pseudolongum
MTNPVIGTPWQKLDRPVSEEAIEGMDKYWRVTNYMSIGQIYLRSNPLMKEPFTRDDVKHRLVGHWGTTPGLNFLLAHINRLIADHQQNTVFIMGPGHGGPAGTSQSYVDGTYTEYYPNITKDEAGLQKFFRQFSYPGGIPSHFAPETPGSIHEGGELGYALSHAYGAVMNNPSLFVPCIIGDGEAETGPLATGWQSNKLVNPRTDGIVLPILHLNGYKIANPTILARISDEELHDFFRGMGYHPYEFVAGFDNEDHMSIHRRFAELFETIFDEICDIKLRPQTDDMTRPFYPMLIFRTPKGWTCPKFIDGKKTEGSWRAHQVPLASARDTEEHFEVLKGWMESYKPEELFNADGSIKDDVTAFMPKGELRIGANPNANGGVIREDLKLPELDQYEVTGVKEYGHGWGQVEAPRALGAYCRDIIKNNPDSFRIFGPDETASNRLNATYEVTDKQWDNGYLSGLVDEHMAVTGQVTEQLSEHQCEGFLEAYLLTGRHGIWSSYESFVHVIDSMLNQHAKWLEATVREIPWRKPISSVNLLVSSHVWRQDHNGFSHQDPGVTSLLINKTFNNDHVTNIYFATDTNMLLAISEKCFKSTNKINAIFAGKQPAPTWVTLDEARAELEAGAAEWKWASNAENNDEVQVVLASAGDVPTQELMAASDALNKMGIKFKVVNVVDLLKLQSRENNDEALTDEEFTELFTADKPVLFAYHSYAQDVRGLIYDRPNHDNFHVVGYKEQGSTTTPFDMVRVNDMDRYALQAAALKLIDADKYADKIDELNAFRKKAFQFAVDNGYDIPEFTDWVYPDVKVDETQMLSATAATAGDNE

SEQ ID NO: 40 - protein, 780 aa, Aspergillus nidulans
MPGEVIERPNPAPKPSHVPDLVEKLIIPAQKTKLEKSDCDALHKYRRAAAYIAAGHWGTCPGLILVYSHLNYLIKKQNLDMLYVVGPGHGAPGLLASLWLEGSLGKFYPQYTKDKEGLHNLISTFSTSAGLPSHINAETPGAIHEGGELGYALSVSFGAVMDNPDLIVTCVVGDGEAETGPTATSWHAIKYIDPAESGAVLPILHVNGFKISERTIFGCMDNREIVCLFTGYGYQVRIVEDLEDIDNDLHSAMSWAVEEIRNIQKAARSGKPIMKPQWPMIVLRTPKGWSGPKELHGQFIEGSFHSHQVPLPNAKKDDEELQALQKWLSSYKPDELFTESGDVIDEILSIIPSDDKKLGMRPEAYKTHLPPDLPDWRQFCVKKGDQFSAMKAIGSFIDQVFVKNPHTVRLFSPDELESNKLSAALSHTGRNFQWDEFSNAKGGRVIEVLSEHLCQGFMQGYTLTGRTGIFPSYESFLGIIHTMMVQYAKFAKMAKETAWHHDVSSINYIETSTWARQEHNGFSHQNPSFIGAVLKLKPYAARVYLPPDANTFLTTLHHCLKSKNYINLMVGSKQPTPVYLSPEEAESHCRAGASIFKFCSTDGGLRPDVVLVGIGVEVMFEVIKAAAILRERCPELRVRVVNVTDLFILENEGAHPHALKHEAFDNLFTEDRSIHFNYHGYVNELQGLLFGRPRLDRATIKGYKEEGSTTTPFDMMLVNEVSRYHVAKAAVTGGARFNEKVKLRHQELCSEFDHNIAETRKYIMNNHQDPEDTYNMPSFN

SEQ ID NO: 41 - protein, 796 aa, Clostridium acetobutylicum
MQSIIGKHKDEGKITPEYLKKIDAYWRAANFISVGQLYLLDNPLLREPLKPEHLKRKVVGHWGTIPGQNFIYAHLNRVIKKYDLDMIYVSGPGHGGQVMVSNSYLDGTYSEVYPNVSRDLNGLKKLCKQFSFPGGISSHMAPETPGSINEGGELGYSLAHSFGAVFDNPDLITACVVGDGEAETGPLATSWQANKFLNPVTDGAVLPILHLNGYKISNPTVLSRIPKDELEKFFEGNGWKPYFVEGEDPEAMHKLMAETLDIVTEEILNIQKNARENNDCSRPKWPMIVLRTPKGWTGPKFVDGVPNEGSFRAHQVPLAVDRYHTENLDQLEEWLKSYKPEELFDENYRLIPELEELTPKGNKRMAANLHANGGLLLRELRTPDFRDYAVDVPTPGSTVKQDMIELGKYVRDVVKLNEDTRNFRIFGPDETMSNRLWAVFEGTKRQWLSEIKEPNDEFLSNDGRIVDSMLSEHLCEGWLEGYLLTGRHGFFASYEAFLRIVDSMITQHGKWLKVTSQLPWRKDIASLNLIATSNVWQQDHNGYTHQDPGLLGHIVDKKPEIVRAYLPADANTLLAVFDKCLHTKHKINLLVTSKHPRQQWLTMDQAVKHVEQGISIWDWASNDKGQEPDVVIASCGDTPTLEALAAVTILHEHLPELKVRFVNVVDMMKLLPENEHPHGLSDKDYNALFTTDKPVIFAFHGFAHLINQLTYHRENRNLHVHGYMEEGTITTPFDMRVQNKLDRFNLVKDVVENLPQLGNRGAHLVQLMNDKLVEHNQYIREVGEDLPEITNWQWHV

SEQ ID NO: 42 - protein, 813 aa, Leuconostoc mesenteroides
MADFDSKEYLELVDKWWRATNYLSAGMIFLKSNPLFSVTNTPIKAEDVKVKPIGHWGTISGQTFLYAHANRLINKYGLNMFYVGGPGHGGQVMVTNAYLDGAYTEDYPEITQDIEGMSHLFKRFSFPGGIGSHMTAQTPGSLHEGGELGYSLSHAFGAVLDNPDQVAFAVVGDGEAETGPSMASWHSIKFLNAKNDGAVLPVLDLNGFKISNPTIFSRMSDEEITKFFEGLGYSPRFIENDDIHDYATYHQLAANILDQAIEDIQAIQNDARENGKYQDGEIPAWPVIIARLPKGWGGPTHDASNNPIENSFRAHQVPLPLEQHDLATLPEFEDWMNSYKPEELFNADGSLKDELKAIAPKGDKRMSANPITNGGADRSDLKLPNWREFANDINDDTRGKEFADSKRNMDMATLSNYLGAVSQLNPTRFRFFGPDETMSNRLWGLFNVTPRQWMEEIKEPQDQLLSPTGRIIDSQLSEHQAEGWLEGYTLTGRVGIFASYESFLRVVDTMVTQHFKWLRHASEQAWRNDYPSLNLIATSTAFQQDHNGYTHQDPGMLTHLAEKKSNFIREYLPADGNSLLAVQERAFSERHKVNLLIASKQPRQQWFTVEEAEVLANEGLKIIDWASTAPSSDVDITFASAGTEPTIETLAALWLINQAFPDVKFRYVNVVELLRLQKKSEPNMNDERELSAEEFNKYFQADTPVIFGFHAYENLIESFFFERKFTGDVYVHGYREDGDITTTYDMRVYSHLDRFHQAKEAAEILSANGKIDQAAADTFIAKMDDTLAKHFQVTRNEGRDIEEFTDWTWSPLK

SEQ ID NO: 43 - protein, 788 aa, Lactobacillus paraplantarum
MTTDYSSPAYLQKVDKYWRAANYLSVGQLYLKDNPLLQQPLKASDVKVHPIGHWGTIAGQNFIYAHLNRVINKYGLKMFYVEGPGHGGQVMVSNSYLDGTYTDIYPEITQDVEGMQKLFKQFSFPGGVASHAAPETPGSIHEGGELGYSISHGVGAILDNPDEIAAVVVGDGESETGPLATSWQSTKFINPINDGAVLPILNLNGFKISNPTIFGRTSDAKIKEYFESMNWEPIFVEGDDPEKVHPALAKAMDEAVEKIKAIQKHARENDDATLPVWPMIVFRAPKGWTGPKSWDGDKIEGSFRAHQIPIPVDQNDMEHADALVDWLESYQPKELFNEDGSLKDDIKEIIPTGDSRMAANPITNGGVDPKALNLPNFRDYAVDTSKEGANVKQDMLVWSDYLRDVIKKNPDNFRLFGPDETMSNRLYGVFETTNRQWMEDIHPDSDQYEAPAGRVLDAQLSEHQAEGWLEGYVLTGRHGLFASYEAFLRVVDSMLTQHFKWLRKANELDWRKKYPSLNIIAASTVFQQDHNGYTHQDPGALTHLAEKKPEYIREYLPADANTLLAVGDVIFRSQEKINYVVTSKHPRQQWFSIEEAKQLVDNGLGIIDWASTDQGSEPDIVFAAAGTEPTLETLAAIQLLHDSFPEMKIRFVNVVDILKLRSPEKDPRGLSDAEFDHYFTKDKPVVFAFHGYEDLVRDIFFDRHNHNLYVHGYRENGDITTPFDVRVMNQMDRFDLAKSAIAAQPAMENTGAAFVQSMDNMLAKHNAYIRDAGTDLPEVNDWQWKGLK

SEQ ID NO: 44 - protein, 796 aa, Lactobacillus plantarum
MSEAIKSKTVDYSSDEYLKRVDEYWRAANYISVGQLYLLNNPLLREPLKATDVKVHPIGHWGTIAGQNFIYAHLNRAINKYGLNMFYIEGPGHGGQVMVSNSYLDGTYTETYPKITQDKAGMKRLFKQFSFPGGVASHADPKTPGSIHEGGELGYSILHGAGAVLDNPGLIAATVVGDGESETGPLATSWQVNKFLNPITDGTVLPILNLNGFKISNPTVLSRESHEELEDYFKGLGWDPHFVEGTDPAKMHKIMAEELDKVIEEIHAIRKNAKDNNDESRPKWPMIVFRAPKGWTGPKSWDGEPIEGSFRAHQIPIPVDRNHMEHADKLVDWLKSYKPEELFDENGTLKPEIAAIIPEGQARMAANPVTNGGKLTKDLITPNIDDYALDNKDHGKEDGSDMTELGKYIRDLIELNKDNKNFRGWGPDETLSNKLGAAFEDTKRQWMEPIHEPNDALLAPQGRIIDSMLSEHMDEGMLEAYNLTGRYGFFASYESFLRVVDSMLTQHFKWLRNSHEETPWRADVPSLNVIASSTAFQQDHNGYSHQDPGIISHLAEKKTEYVRAYLPGDANTLIATFDKAIQSKQLINLIIASKHPRPQWFTMDEAKRLVRDGLGVIDWASTDHGEEPDVVFATAGSEPTTESLAAVSILHARFPEMKIRFINVVDLLKLKKDDPRGLSDAEFDAFFTKDKPVIFAYHAYDDLVKTIFFDRHNHNLHVHGYREEGDITTPFDMRVRNELDRFHLVKAALLATPAYAEKGAHVIQEMNSILDKHHDYIRAEGTDIPEVENWKWTALK